European Patent Application EP 4 386 004 A1, published June 19, 2024. Title: Anti-VEGF A and anti-VEGF C bispecific antibodies and uses thereof. Applicant: INNOVENT BIOLOGICS (SUZHOU) CO., LTD. The sequence listing filed with the application follows.

SEQUENCE LISTING (53 sequences)

SEQ ID NO: 1 - protein, 10 aa, synthetic construct
GSMFSMYAMG

SEQ ID NO: 2 - protein, 16 aa, synthetic construct
ATTSGGSTLYADSVKG

SEQ ID NO: 3 - protein, 10 aa, synthetic construct
YWRGSDPENY

SEQ ID NO: 4 - protein, 118 aa, synthetic construct
QLQLVESGGGLVQPGGSLRLSCAASGSMFSMYAMGWYRQAPGKQRELVAATTSGGSTLYADSVKGRFTISRDNAENTVYLQMNSLKPEDTAVYYCYTYWRGSDPENYWGRGTQVTVSS

SEQ ID NO: 5 - protein, 10 aa, synthetic construct
GSMFSMYAMG

SEQ ID NO: 6 - protein, 16 aa, synthetic construct
ATTSGGSTLYADSVKG

SEQ ID NO: 7 - protein, 10 aa, synthetic construct
YWRGSDPENY

SEQ ID NO: 8 - protein, 118 aa, synthetic construct
EVQLVESGGGLVQPGGSLRLSCAASGSMFSMYAMGWYRQAPGKQRELVAATTSGGSTLYADSVKGRFTISRDNSKNTLYLQMNSLRAEDTAVYYCYTYWRGSDPENYWGQGTQVTVSS

SEQ ID NO: 9 - protein, 10 aa, synthetic construct
GSSFSPYAMG

SEQ ID NO: 10 - protein, 16 aa, synthetic construct
ATTSGGSTLYADSVKG

SEQ ID NO: 11 - protein, 10 aa, synthetic construct
HWRGSDPENY

SEQ ID NO: 12 - protein, 118 aa, synthetic construct
QLQLVESGGGLVQPGGSLRLSCAASGSSFSPYAMGWYRQAPGKQRELVAATTSGGSTLYADSVKGRFTISRDNAKNTVYLQMNSLKPEDTAVYYCYMHWRGSDPENYWGQGTQVTVSS

SEQ ID NO: 13 - protein, 10 aa, synthetic construct
GSSFSPYAMG

SEQ ID NO: 14 - protein, 16 aa, synthetic construct
ATTSGGSTLYADSVKG

SEQ ID NO: 15 - protein, 10 aa, synthetic construct
HWRGSDPENY

SEQ ID NO: 16 - protein, 118 aa, synthetic construct
EVQLVESGGGLVQPGGSLRLSCAASGSSFSPYAMGWYRQAPGKQRELVSATTSGGSTLYADSVKGRFTISRDNSKNTVYLQMNSLRAEDTAVYYCYMHWRGSDPENYWGQGTQVTVSS

SEQ ID NO: 17 - protein, 10 aa, synthetic construct
GSSFSPYAMG

SEQ ID NO: 18 - protein, 16 aa, synthetic construct
ATSEGGFTLYADSVKG

SEQ ID NO: 19 - protein, 10 aa, synthetic construct
HWRGSDPENY

SEQ ID NO: 20 - protein, 118 aa, synthetic construct
EVQLVESGGGLVQPGGSLRLSCAASGSSFSPYAMGWYRQAPGKQRELVSATSEGGFTLYADSVKGRFTISRDNSKNTVYLQMNSLRAEDTAVYYCYMHWRGSDPENYWGQGTQVTVSS

SEQ ID NO: 21 - protein, 10 aa, synthetic construct
GSSFSPYAMG

SEQ ID NO: 22 - protein, 16 aa, synthetic construct
ATSSGGFTLYADSVKG

SEQ ID NO: 23 - protein, 10 aa, synthetic construct
YYREYDPEMY

SEQ ID NO: 24 - protein, 118 aa, synthetic construct
EVQLVESGGGLVQPGGSLRLSCAASGSSFSPYAMGWYRQAPGKQRELVSATSSGGFTLYADSVKGRFTISRDNSKNTVYLQMNSLRAEDTAVYYCYTYYREYDPEMYWGQGTQVTVSS

SEQ ID NO: 25 - protein, 431 aa, synthetic construct
SDTGRPFVEMYSEIPEIIHMTEGRELVIPCRVTSPNITVTLKKFPLDTLIPDGKRIIWDSRKGFIISNATYKEIGLLTCEATVNGHLYKTNYLTHRQTNTIIDVVLSPSHGIELSVGEKLVLNCTARTELNVGIDFNWEYPSSKHQHKKLVNRDLKTQSGSEMKKFLSTLTIDGVTRSDQGLYTCAASSGLMTKKNSTFVRVHEKDKTHTCPPCPAPELLGGPSVFLFPPKPKDTLMISRTPEVTCVVVDVSHEDPEVKFNWYVDGVEVHNAKTKPREEQYNSTYRVVSVLTVLHQDWLNGKEYKCKVSNKALPAPIEKTISKAKGQPREPQVYTLPPSRDELTKNQVSLTCLVKGFYPSDIAVEWESNGQPENNYKTTPPVLDSDGSFFLYSKLTVDKSRWQQGNVFSCSVMHEALHNHYTQKSLSLSPG

SEQ ID NO: 26 - protein, 205 aa, synthetic construct
SDTGRPFVEMYSEIPEIIHMTEGRELVIPCRVTSPNITVTLKKFPLDTLIPDGKRIIWDSRKGFIISNATYKEIGLLTCEATVNGHLYKTNYLTHRQTNTIIDVVLSPSHGIELSVGEKLVLNCTARTELNVGIDFNWEYPSSKHQHKKLVNRDLKTQSGSEMKKFLSTLTIDGVTRSDQGLYTCAASSGLMTKKNSTFVRVHEK

SEQ ID NO: 27 - protein, 226 aa, synthetic construct
DKTHTCPPCPAPELLGGPSVFLFPPKPKDTLMISRTPEVTCVVVDVSHEDPEVKFNWYVDGVEVHNAKTKPREEQYNSTYRVVSVLTVLHQDWLNGKEYKCKVSNKALPAPIEKTISKAKGQPREPQVYTLPPSRDELTKNQVSLTCLVKGFYPSDIAVEWESNGQPENNYKTTPPVLDSDGSFFLYSKLTVDKSRWQQGNVFSCSVMHEALHNHYTQKSLSLSPG

SEQ ID NO: 28 - protein, 231 aa, synthetic construct
EVQLVESGGGLVQPGGSLRLSCAASGYDFTHYGMNWVRQAPGKGLEWVGWINTYTGEPTYAADFKRRFTFSLDTSKSTAYLQMNSLRAEDTAVYYCAKYPYYYGTSHWYFDVWGQGTLVTVSSASTKGPSVFPLAPSSKSTSGGTAALGCLVKDYFPEPVTVSWNSGALTSGVHTFPAVLQSSGLYSLSSVVTVPSSSLGTQTYICNVNHKPSNTKVDKKVEPKSCDKTHL

SEQ ID NO: 29 - protein, 123 aa, synthetic construct [sequence omitted]

SEQ ID NO: 30 - protein, 108 aa, synthetic construct
ASTKGPSVFPLAPSSKSTSGGTAALGCLVKDYFPEPVTVSWNSGALTSGVHTFPAVLQSSGLYSLSSVVTVPSSSLGTQTYICNVNHKPSNTKVDKKVEPKSCDKTHL

SEQ ID NO: 31 - protein, 214 aa, synthetic construct
DIQLTQSPSSLSASVGDRVTITCSASQDISNYLNWYQQKPGKAPKVLIYFTSSLHSGVPSRFSGSGSGTDFTLTISSLQPEDFATYYCQQYSTVPWTFGQGTKVEIKRTVAAPSVFIFPPSDEQLKSGTASVVCLLNNFYPREAKVQWKVDNALQSGNSQESVTEQDSKDSTYSLSSTLTLSKADYEKHKVYACEVTHQGLSSPVTKSFNRGEC

SEQ ID NO: 32 - protein, 107 aa, synthetic construct [sequence omitted]

SEQ ID NO: 33 - protein, 107 aa, synthetic construct [sequence omitted]

SEQ ID NO: 34 - protein, 7 aa, synthetic construct
GYDFTHY

SEQ ID NO: 35 - protein, 6 aa, synthetic construct
NTYTGE

SEQ ID NO: 36 - protein, 14 aa, synthetic construct
YPYYYGTSHWYFDV

SEQ ID NO: 37 - protein, 8 aa, synthetic construct
QDISNYLN

SEQ ID NO: 38 - protein, 7 aa, synthetic construct
FTSSLHS

SEQ ID NO: 39 - protein, 9 aa, synthetic construct
QQYSTVPWT

SEQ ID NO: 40 - protein, 564 aa, synthetic construct
SDTGRPFVEMYSEIPEIIHMTEGRELVIPCRVTSPNITVTLKKFPLDTLIPDGKRIIWDSRKGFIISNATYKEIGLLTCEATVNGHLYKTNYLTHRQTNTIIDVVLSPSHGIELSVGEKLVLNCTARTELNVGIDFNWEYPSSKHQHKKLVNRDLKTQSGSEMKKFLSTLTIDGVTRSDQGLYTCAASSGLMTKKNSTFVRVHEKDKTHTCPPCPAPELLGGPSVFLFPPKPKDTLMISRTPEVTCVVVDVSHEDPEVKFNWYVDGVEVHNAKTKPREEQYNSTYRVVSVLTVLHQDWLNGKEYKCKVSNKALPAPIEKTISKAKGQPREPQVYTLPPSRDELTKNQVSLTCLVKGFYPSDIAVEWESNGQPENNYKTTPPVLDSDGSFFLYSKLTVDKSRWQQGNVFSCSVMHEALHNHYTQKSLSLSPGGGGGSGGGGSGGGGSQLQLVESGGGLVQPGGSLRLSCAASGSSFSPYAMGWYRQAPGKQRELVAATTSGGSTLYADSVKGRFTISRDNAKNTVYLQMNSLKPEDTAVYYCYMHWRGSDPENYWGQGTQVTVSS

SEQ ID NO: 41 - protein, 564 aa, synthetic construct
SDTGRPFVEMYSEIPEIIHMTEGRELVIPCRVTSPNITVTLKKFPLDTLIPDGKRIIWDSRKGFIISNATYKEIGLLTCEATVNGHLYKTNYLTHRQTNTIIDVVLSPSHGIELSVGEKLVLNCTARTELNVGIDFNWEYPSSKHQHKKLVNRDLKTQSGSEMKKFLSTLTIDGVTRSDQGLYTCAASSGLMTKKNSTFVRVHEKDKTHTCPPCPAPELLGGPSVFLFPPKPKDTLMISRTPEVTCVVVDVSHEDPEVKFNWYVDGVEVHNAKTKPREEQYNSTYRVVSVLTVLHQDWLNGKEYKCKVSNKALPAPIEKTISKAKGQPREPQVYTLPPSRDELTKNQVSLTCLVKGFYPSDIAVEWESNGQPENNYKTTPPVLDSDGSFFLYSKLTVDKSRWQQGNVFSCSVMHEALHNHYTQKSLSLSPGGGGGSGGGGSGGGGSEVQLVESGGGLVQPGGSLRLSCAASGSSFSPYAMGWYRQAPGKQRELVSATTSGGSTLYADSVKGRFTISRDNSKNTVYLQMNSLRAEDTAVYYCYMHWRGSDPENYWGQGTQVTVSS

SEQ ID NO: 42 - protein, 364 aa, synthetic construct
EVQLVESGGGLVQPGGSLRLSCAASGYDFTHYGMNWVRQAPGKGLEWVGWINTYTGEPTYAADFKRRFTFSLDTSKSTAYLQMNSLRAEDTAVYYCAKYPYYYGTSHWYFDVWGQGTLVTVSSASTKGPSVFPLAPSSKSTSGGTAALGCLVKDYFPEPVTVSWNSGALTSGVHTFPAVLQSSGLYSLSSVVTVPSSSLGTQTYICNVNHKPSNTKVDKKVEPKSCDKTHLGGGGSGGGGSGGGGSEVQLVESGGGLVQPGGSLRLSCAASGSSFSPYAMGWYRQAPGKQRELVSATTSGGSTLYADSVKGRFTISRDNSKNTVYLQMNSLRAEDTAVYYCYMHWRGSDPENYWGQGTQVTVSS

SEQ ID NO: 43 - protein, 347 aa, synthetic construct
DIQLTQSPSSLSASVGDRVTITCSASQDISNYLNWYQQKPGKAPKVLIYFTSSLHSGVPSRFSGSGSGTDFTLTISSLQPEDFATYYCQQYSTVPWTFGQGTKVEIKRTVAAPSVFIFPPSDEQLKSGTASVVCLLNNFYPREAKVQWKVDNALQSGNSQESVTEQDSKDSTYSLSSTLTLSKADYEKHKVYACEVTHQGLSSPVTKSFNRGECGGGGSGGGGSGGGGSEVQLVESGGGLVQPGGSLRLSCAASGSSFSPYAMGWYRQAPGKQRELVSATTSGGSTLYADSVKGRFTISRDNSKNTVYLQMNSLRAEDTAVYYCYMHWRGSDPENYWGQGTQVTVSS

SEQ ID NO: 44 - protein, 559 aa, synthetic construct
SDTGRPFVEMYSEIPEIIHMTEGRELVIPCRVTSPNITVTLKKFPLDTLIPDGKRIIWDSRKGFIISNATYKEIGLLTCEATVNGHLYKTNYLTHRQTNTIIDVVLSPSHGIELSVGEKLVLNCTARTELNVGIDFNWEYPSSKHQHKKLVNRDLKTQSGSEMKKFLSTLTIDGVTRSDQGLYTCAASSGLMTKKNSTFVRVHEKDKTHTCPPCPAPELLGGPSVFLFPPKPKDTLMISRTPEVTCVVVDVSHEDPEVKFNWYVDGVEVHNAKTKPREEQYNSTYRVVSVLTVLHQDWLNGKEYKCKVSNKALPAPIEKTISKAKGQPREPQVYTLPPSRDELTKNQVSLTCLVKGFYPSDIAVEWESNGQPENNYKTTPPVLDSDGSFFLYSKLTVDKSRWQQGNVFSCSVMHEALHNHYTQKSLSLSPGGGGGSGGGGSEVQLVESGGGLVQPGGSLRLSCAASGSSFSPYAMGWYRQAPGKQRELVSATTSGGSTLYADSVKGRFTISRDNSKNTVYLQMNSLRAEDTAVYYCYMHWRGSDPENYWGQGTQVTVSS

SEQ ID NO: 45 - protein, 569 aa, synthetic construct
SDTGRPFVEMYSEIPEIIHMTEGRELVIPCRVTSPNITVTLKKFPLDTLIPDGKRIIWDSRKGFIISNATYKEIGLLTCEATVNGHLYKTNYLTHRQTNTIIDVVLSPSHGIELSVGEKLVLNCTARTELNVGIDFNWEYPSSKHQHKKLVNRDLKTQSGSEMKKFLSTLTIDGVTRSDQGLYTCAASSGLMTKKNSTFVRVHEKDKTHTCPPCPAPELLGGPSVFLFPPKPKDTLMISRTPEVTCVVVDVSHEDPEVKFNWYVDGVEVHNAKTKPREEQYNSTYRVVSVLTVLHQDWLNGKEYKCKVSNKALPAPIEKTISKAKGQPREPQVYTLPPSRDELTKNQVSLTCLVKGFYPSDIAVEWESNGQPENNYKTTPPVLDSDGSFFLYSKLTVDKSRWQQGNVFSCSVMHEALHNHYTQKSLSLSPGGGGGSGGGGSGGGGSGGGGSEVQLVESGGGLVQPGGSLRLSCAASGSSFSPYAMGWYRQAPGKQRELVSATTSGGSTLYADSVKGRFTISRDNSKNTVYLQMNSLRAEDTAVYYCYMHWRGSDPENYWGQGTQVTVSS

SEQ ID NO: 46 - protein, 564 aa, synthetic construct
SDTGRPFVEMYSEIPEIIHMTEGRELVIPCRVTSPNITVTLKKFPLDTLIPDGKRIIWDSRKGFIISNATYKEIGLLTCEATVNGHLYKTNYLTHRQTNTIIDVVLSPSHGIELSVGEKLVLNCTARTELNVGIDFNWEYPSSKHQHKKLVNRDLKTQSGSEMKKFLSTLTIDGVTRSDQGLYTCAASSGLMTKKNSTFVRVHEKDKTHTCPPCPAPELLGGPSVFLFPPKPKDTLMISRTPEVTCVVVDVSHEDPEVKFNWYVDGVEVHNAKTKPREEQYNSTYRVVSVLTVLHQDWLNGKEYKCKVSNKALPAPIEKTISKAKGQPREPQVYTLPPSRDELTKNQVSLTCLVKGFYPSDIAVEWESNGQPENNYKTTPPVLDSDGSFFLYSKLTVDKSRWQQGNVFSCSVMHEALHNHYTQKSLSLSPGGGGGSGGGGSGGGGSEVQLVESGGGLVQPGGSLRLSCAASGSSFSPYAMGWYRQAPGKQRELVSATSEGGFTLYADSVKGRFTISRDNSKNTVYLQMNSLRAEDTAVYYCYMHWRGSDPENYWGQGTQVTVSS

SEQ ID NO: 47 - protein, 564 aa, synthetic construct
SDTGRPFVEMYSEIPEIIHMTEGRELVIPCRVTSPNITVTLKKFPLDTLIPDGKRIIWDSRKGFIISNATYKEIGLLTCEATVNGHLYKTNYLTHRQTNTIIDVVLSPSHGIELSVGEKLVLNCTARTELNVGIDFNWEYPSSKHQHKKLVNRDLKTQSGSEMKKFLSTLTIDGVTRSDQGLYTCAASSGLMTKKNSTFVRVHEKDKTHTCPPCPAPELLGGPSVFLFPPKPKDTLMISRTPEVTCVVVDVSHEDPEVKFNWYVDGVEVHNAKTKPREEQYNSTYRVVSVLTVLHQDWLNGKEYKCKVSNKALPAPIEKTISKAKGQPREPQVYTLPPSRDELTKNQVSLTCLVKGFYPSDIAVEWESNGQPENNYKTTPPVLDSDGSFFLYSKLTVDKSRWQQGNVFSCSVMHEALHNHYTQKSLSLSPGGGGGSGGGGSGGGGSEVQLVESGGGLVQPGGSLRLSCAASGSSFSPYAMGWYRQAPGKQRELVSATSSGGFTLYADSVKGRFTISRDNSKNTVYLQMNSLRAEDTAVYYCYTYYREYDPEMYWGQGTQVTVSS

SEQ ID NO: 48 - protein, 364 aa, synthetic construct
EVQLVESGGGLVQPGGSLRLSCAASGYDFTHYGMNWVRQAPGKGLEWVGWINTYTGEPTYAADFKRRFTFSLDTSKSTAYLQMNSLRAEDTAVYYCAKYPYYYGTSHWYFDVWGQGTLVTVSSASTKGPSVFPLAPSSKSTSGGTAALGCLVKDYFPEPVTVSWNSGALTSGVHTFPAVLQSSGLYSLSSVVTVPSSSLGTQTYICNVNHKPSNTKVDKKVEPKSCDKTHLGGGGSGGGGSGGGGSEVQLVESGGGLVQPGGSLRLSCAASGSSFSPYAMGWYRQAPGKQRELVSATSEGGFTLYADSVKGRFTISRDNSKNTVYLQMNSLRAEDTAVYYCYMHWRGSDPENYWGQGTQVTVSS

SEQ ID NO: 49 - protein, 347 aa, synthetic construct
DIQLTQSPSSLSASVGDRVTITCSASQDISNYLNWYQQKPGKAPKVLIYFTSSLHSGVPSRFSGSGSGTDFTLTISSLQPEDFATYYCQQYSTVPWTFGQGTKVEIKRTVAAPSVFIFPPSDEQLKSGTASVVCLLNNFYPREAKVQWKVDNALQSGNSQESVTEQDSKDSTYSLSSTLTLSKADYEKHKVYACEVTHQGLSSPVTKSFNRGECGGGGSGGGGSGGGGSEVQLVESGGGLVQPGGSLRLSCAASGSSFSPYAMGWYRQAPGKQRELVSATSEGGFTLYADSVKGRFTISRDNSKNTVYLQMNSLRAEDTAVYYCYMHWRGSDPENYWGQGTQVTVSS

SEQ ID NO: 50 - protein, 364 aa, synthetic construct
EVQLVESGGGLVQPGGSLRLSCAASGYDFTHYGMNWVRQAPGKGLEWVGWINTYTGEPTYAADFKRRFTFSLDTSKSTAYLQMNSLRAEDTAVYYCAKYPYYYGTSHWYFDVWGQGTLVTVSSASTKGPSVFPLAPSSKSTSGGTAALGCLVKDYFPEPVTVSWNSGALTSGVHTFPAVLQSSGLYSLSSVVTVPSSSLGTQTYICNVNHKPSNTKVDKKVEPKSCDKTHLGGGGSGGGGSGGGGSEVQLVESGGGLVQPGGSLRLSCAASGSSFSPYAMGWYRQAPGKQRELVSATSSGGFTLYADSVKGRFTISRDNSKNTVYLQMNSLRAEDTAVYYCYTYYREYDPEMYWGQGTQVTVSS

SEQ ID NO: 51 - protein, 347 aa, synthetic construct
DIQLTQSPSSLSASVGDRVTITCSASQDISNYLNWYQQKPGKAPKVLIYFTSSLHSGVPSRFSGSGSGTDFTLTISSLQPEDFATYYCQQYSTVPWTFGQGTKVEIKRTVAAPSVFIFPPSDEQLKSGTASVVCLLNNFYPREAKVQWKVDNALQSGNSQESVTEQDSKDSTYSLSSTLTLSKADYEKHKVYACEVTHQGLSSPVTKSFNRGECGGGGSGGGGSGGGGSEVQLVESGGGLVQPGGSLRLSCAASGSSFSPYAMGWYRQAPGKQRELVSATSSGGFTLYADSVKGRFTISRDNSKNTVYLQMNSLRAEDTAVYYCYTYYREYDPEMYWGQGTQVTVSS

SEQ ID NO: 52 - protein, 537 aa, synthetic construct
YSMTPPTLNITEESHVIDTGDSLSISCRGQHPLEWAWPGAQEAPATGDKDSEDTGVVRDCEGTDARPYCKVLLLHEVHAQDTGSYVCYYKYIKARIEGTTAASSYVFVRDFEQPFINKPDTLLVNRKDAMWVPCLVSIPGLNVTLRSQSSVLWPDGQEVVWDDRRGMLVSTPLLHDALYLQCETTWGDQDFLSNPFLVHITGNELYDIQLLPRKSLELLVGEKLVLNCTVWAEFNSGVTFDWDYPGKQAERGKWVPERRSQQTHTELSSILTIHNVSQHDLGSYVCKANNGIQRFRESTEVIVHEEPKSCDKTHTCPPCPAPELLGGPSVFLFPPKPKDTLMISRTPEVTCVVVDVSHEDPEVKFNWYVDGVEVHNAKTKPREEQYNSTYRVVSVLTVLHQDWLNGKEYKCKVSNKALPAPIEKTISKAKGQPREPQVYTLPPSRDELTKNQVSLTCLVKGFYPSDIAVEWESNGQPENNYKTTPPVLDSDGSFFLYSKLTVDKSRWQQGNVFSCSVMHEALHNHYTQKSLSLSPGK

SEQ ID NO: 53 - protein, 434 aa, synthetic construct
PFVEMYSEIPEIIHMTEGRELVIPCRVTSPNITVTLKKFPLDTLIPDGKRIIWDSRKGFIISNATYKEIGLLTCEATVNGHLYKTNYLTHRQTVVLSPSHGIELSVGEKLVLNCTARTELNVGIDFNWEYPSSKHQHKKLVNRDLKTQSGSEMKKFLSTLTIDGVTRSDQGLYTCAASSGLMTKKNSTFVRVHEKGGGGGGGGGGGGDKTHTCPLCPAPELLGGPSVFLFPPKPKDTLMISRTPEVTCVVVDVSHEDPEVKFNWYVDGVEVHNAKTKPREEQYNSTYRVVSVLTVLHQDWLNGKEYKCKVSNKALPAPIEKTISKAKGQPREPQVYTLPPSRDELTKNQVSLTCLVKGFYPSDIAVEWESNGQPENNYKATPPVLDSDGSFFLYSKLTVDKSRWQQGNVFSCSVMHEALHNHYTQKSLSLSPGK